European Patent Specification EP 3 414 263 B1, published April 5, 2023. Title: SIGNALLING SYSTEM. Applicant: Autolus Ltd. The sequence listing filed with the application follows.

SEQUENCE LISTING (37 sequences)

SEQ ID NO: 1 - protein, 112 aa, Artificial Sequence
  CD3 Z endodomain
RVKFSRSADAPAYQQGQNQLYNELNLGRREEYDVLDKRRGRDPEMGGKPRRKNPQEGLYNELQKDKMAEAYSEIGMKGERRRGKGHDGLYQGLSTATKDTYDALHMQALPPR

SEQ ID NO: 2 - protein, 152 aa, Artificial Sequence
  CD28 and CD3 Zeta endodomains
SKRSRLLHSDYMNMTPRRPGPTRKHYQPYAPPRDFAAYRSRVKFSRSADAPAYQQGQNQLYNELNLGRREEYDVLDKRRGRDPEMGGKPRRKNPQEGLYNELQKDKMAEAYSEIGMKGERRRGKGHDGLYQGLSTATKDTYDALHMQALPPR

SEQ ID NO: 3 - protein, 188 aa, Artificial Sequence
  CD28, OX40 and CD3 Zeta endodomains
SKRSRLLHSDYMNMTPRRPGPTRKHYQPYAPPRDFAAYRSRDQRLPPDAHKPPGGGSFRTPIQEEQADAHSTLAKIRVKFSRSADAPAYQQGQNQLYNELNLGRREEYDVLDKRRGRDPEMGGKPRRKNPQEGLYNELQKDKMAEAYSEIGMKGERRRGKGHDGLYQGLSTATKDTYDALHMQALPPR

SEQ ID NO: 4 - protein, 20 aa, Foot-and-mouth disease virus
RAEGRGSLLTCGDVEENPGP

SEQ ID NO: 5 - protein, 20 aa, Foot-and-mouth disease virus
QCTNYALLKLAGDVESNPGP

SEQ ID NO: 6 - protein, 10 aa, Artificial Sequence
  single domain binder-interacting peptide (sdbiP) which binds a methotrexate dAb
ACNAGHLSQC

SEQ ID NO: 7 - protein, 7 aa, Artificial Sequence
  sdbiP which binds a methotrexate dAb
ASLAITH

SEQ ID NO: 8 - protein, 10 aa, Artificial Sequence
  sdbiP which binds a methotrexate dAb
ACISLTLNRC

SEQ ID NO: 9 - protein, 7 aa, Artificial Sequence
  sdbiP which binds a methotrexate dAb
QTEKNPL

SEQ ID NO: 10 - protein, 10 aa, Artificial Sequence
  sdbiP which binds a methotrexate dAb
ACNAGHLSQC

SEQ ID NO: 11 - protein, 119 aa, Artificial Sequence
  caffeine single domain binder
EVQLQASGGGLVQAGGSLRLSCTASGRTGTIYSMAWFRQAPGKEREFLATVGWSSGITYYMDSVKGRFTISRDNAKNSAYLQMNSLKPEDTAVYYCTATRAYSVGYDYWGQGTQVTVSS

SEQ ID NO: 12 - protein, 7 aa, Artificial Sequence
  sdbiP which binds a caffeine dAb
HTLNKPP

SEQ ID NO: 13 - protein, 7 aa, Artificial Sequence
  sdbiP which binds a caffeine dAb
DLSIGNH

SEQ ID NO: 14 - protein, 7 aa, Artificial Sequence
  sdbiP which binds a caffeine dAb
HDSPTAA

SEQ ID NO: 15 - protein, 7 aa, Artificial Sequence
  sdbiP which binds a caffeine dAb
YPDVPLA

SEQ ID NO: 16 - protein, 10 aa, Artificial Sequence
  sdbiP which binds a caffeine dAb
ACTYLNSAKC

SEQ ID NO: 17 - protein, 8 aa, Artificial Sequence
  complementarity determining region (CDR), CDR1
GRTFSSYN

SEQ ID NO: 18 - protein, 8 aa, Artificial Sequence
  CDR2
ISWSGART

SEQ ID NO: 19 - protein, 14 aa, Artificial Sequence
  CDR3
AAGRGWGTEAILDY

SEQ ID NO: 20 - protein, 8 aa, Artificial Sequence
  CDR1
GRSLSSYV

SEQ ID NO: 21 - protein, 14 aa, Artificial Sequence
  CDR3
VAGRGWGTEAILDY

SEQ ID NO: 22 - protein, 8 aa, Artificial Sequence
  CDR1
GRTFSNYN

SEQ ID NO: 23 - protein, 8 aa, Artificial Sequence
  CDR2
INWSGGRT

SEQ ID NO: 24 - protein, 8 aa, Artificial Sequence
  CDR1
GRTFSRYN

SEQ ID NO: 25 - protein, 8 aa, Artificial Sequence
  CDR2
ISRSGGIT

SEQ ID NO: 26 - protein, 14 aa, Artificial Sequence
  CDR3
AAGRGWGVEAILDY

SEQ ID NO: 27 - protein, 8 aa, Artificial Sequence
  CDR1
GNIGLVSV

SEQ ID NO: 28 - protein, 7 aa, Artificial Sequence
  CDR2
ITGGGST

SEQ ID NO: 29 - protein, 9 aa, Artificial Sequence
  CDR3
RLVNNGRPF

SEQ ID NO: 30 - protein, 9 aa, Artificial Sequence
  CDR1
GRLSLSSYV

SEQ ID NO: 31 - protein, 6 aa, Artificial Sequence
  Caffeine dAb CDR1
TIYSMA

SEQ ID NO: 32 - protein, 17 aa, Artificial Sequence
  Caffeine dAb CDR2
TVGWSSGITYYMDSVKG

SEQ ID NO: 33 - protein, 10 aa, Artificial Sequence
  Caffeine dAb CDR3
TRAYSVGYDY

SEQ ID NO: 34 - protein, 16 aa, Artificial Sequence
  TetR interacting peptide (TiP)
WTWNAYAFAAPSGGGS

SEQ ID NO: 35 - protein, 87 aa, Artificial Sequence
  intracellular linker domain derived from CD4 (WT)
LSDSGQVLLESNIKVLPTWSTPVQPMALIVLGGVAGLLLFIGLGIFFCVRCRHRRRQAERMSQIKRLLSEKKTCQCPHRFQKTCSPI

SEQ ID NO: 36 - protein, 61 aa, Artificial Sequence
  CD4 endodomain optimized for
ALIVLGGVAGLLLFIGLGIFFCVRCRHRRRQAERMAQIKRVVSEKKTAQAPHRFQKTCSPI

SEQ ID NO: 37 - protein, 926 aa, Artificial Sequence
  TetCAR amino acid sequence
MWTWNAYAFAAPSGGGSADAPAYQQGQNQLYNELNLGRREEYDVLDKRRGRDPEMGGKPRRKNPQEGLYNELQKDKMAEAYSEIGMKGERRRGKGHDGLYQGLSTATKDTYDALHMQALPPRRAEGRGSLLTCGDVEENPGPMAVPTQVLGLLLLWLTDARCDIQMTQSPSSLSASVGDRVTITCRASEDIYFNLVWYQQKPGKAPKLLIYDTNRLADGVPSRFSGSGSGTQYTLTISSLQPEDFATYYCQHYKNYPLTFGQGTKLEIKRSGGGGSGGGGSGGGGSGGGGSRSEVQLVESGGGLVQPGGSLRLSCAASGFTLSNYGMHWIRQAPGKGLEWVSSISLNGGSTYYRDSVKGRFTISRDNAKSTLYLQMNSLRAEDTAVYYCAAQDAYTGGYFDYWGQGTLVTVSSMDPAEPKSPDKTHTCPPCPAPPVAGPSVFLFPPKPKDTLMIARTPEVTCVVVDVSHEDPEVKFNWYVDGVEVHNAKTKPREEQYNSTYRVVSVLTVLHQDWLNGKEYKCKVSNKALPAPIEKTISKAKGQPREPQVYTLPPSRDELTKNQVSLTCLVKGFYPSDIAVEWESNGQPENNYKTTPPVLDSDGSFFLYSKLTVDKSRWQQGNVFSCSVMHEALHNHYTQKSLSLSPGKKDPMALIVLGGVAGLLLFIGLGIFFCVRCRHRRRQAERMAQIKRVVSEKKTAQAPHRFQKTCSPISGGGGSMSRLDKSKVINSALELLNEVGIEGLTTRKLAQKLGVEQPTLYWHVKNKRALLDALAIEMLDRHHTHFCPLEGESWQDFLRNNAKSFRCALLSHRDGAKVHLGTRPTEKQYETLENQLAFLCQQGFSLENALYALSAVGHFTLGCVLEDQEHQVAKEERETPTTDSMPPLLRQAIELFDHQGAEPAFLFGLELIICGLEKQLKCESGS